European Patent Application EP 4 806 905 A1, published September 16, 2026. Title: PEPTIDE, PEPTIDE COMPLEX, PHARMACEUTICAL COMPOSITION, CELL CULTURE COMPOSITION, AND COMPOSITION FOR USE IN MEDICAL, DIAGNOSIS OR RESEARCH. Applicant: ペプチドリーム株式会社. Application JP. The sequence listing filed with the application follows.

SEQUENCE LISTING (165 sequences)

SEQ ID NO: 1 - protein, 15 aa, unidentified
  SITE 1: note = D-phenylalanine
  SITE 7: note = Methyl-L-phenylalanine
  SITE 10: note = Methyl-L-phenylalanine
XSDIRYXQTXIVGCG

SEQ ID NO: 2 - protein, 15 aa, unidentified
  SITE 1: note = (R)-2-amino-5-ureidopentanoic acid
  SITE 7: note = Methyl-L-phenylalanine
  SITE 10: note = Methyl-L-phenylalanine
XSDIRYXQTXIVGCG

SEQ ID NO: 3 - protein, 15 aa, unidentified
  SITE 1: note = D-tyrosine
  SITE 7: note = Methyl-L-phenylalanine
  SITE 10: note = Methyl-L-phenylalanine
XSDIRYXQTXIVGCG

SEQ ID NO: 4 - protein, 15 aa, unidentified
  SITE 1: note = (R)-2-amino-3-(4-fluorophenyl)propanoic acid
  SITE 7: note = Methyl-L-phenylalanine
  SITE 10: note = Methyl-L-phenylalanine
XSDIRYXQTXIVGCG

SEQ ID NO: 5 - protein, 15 aa, unidentified
  SITE 1: note = D-phenylalanine
  SITE 6: note = Methyl-L-tyrosine
  SITE 7: note = Methyl-L-phenylalanine
  SITE 10: note = Methyl-L-phenylalanine
XSDIRXXQTXIVGCG

SEQ ID NO: 6 - protein, 15 aa, unidentified
  SITE 1: note = D-phenylalanine
  SITE 7: note = Methyl-L-phenylalanine
  SITE 10: note = Methyl-L-phenylalanine
  SITE 12: note = Methyl-L-valine
XSDIRYXQTXIXGCG

SEQ ID NO: 7 - protein, 15 aa, unidentified
  SITE 1: note = D-phenylalanine
  SITE 7: note = Methyl-L-phenylalanine
  SITE 10: note = Methyl-L-phenylalanine
  SITE 12: note = Methyl-L-valine
XSDIRYXVTXIXGCG

SEQ ID NO: 8 - protein, 15 aa, unidentified
  SITE 1: note = D-phenylalanine
  SITE 2: note = (S)-2-amino-6-morpholinohexanoic acid
  SITE 7: note = Methyl-L-phenylalanine
  SITE 10: note = Methyl-L-phenylalanine
XXDIRYXQTXIVGCG

SEQ ID NO: 9 - protein, 15 aa, unidentified
  SITE 1: note = D-phenylalanine
  SITE 7: note = Methyl-L-phenylalanine
  SITE 10: note = Methyl-L-phenylalanine
XSRIRYXQTXIVGCG

SEQ ID NO: 10 - protein, 15 aa, unidentified
  SITE 1: note = D-phenylalanine
  SITE 3: note = L-citrulline
  SITE 7: note = Methyl-L-phenylalanine
  SITE 10: note = Methyl-L-phenylalanine
XSXIRYXQTXIVGCG

SEQ ID NO: 11 - protein, 15 aa, unidentified
  SITE 1: note = D-phenylalanine
  SITE 3: note = N6-(4-(carboxymethyl)piperazine-1-carbonyl)-L-lysine
  SITE 7: note = Methyl-L-phenylalanine
  SITE 10: note = Methyl-L-phenylalanine
XSXIRYXQTXIVGCG

SEQ ID NO: 12 - protein, 15 aa, unidentified
  SITE 1: note = D-phenylalanine
  SITE 3: note = (2S)-2-amino-3-(oxan-4-yl)propanoic acid
  SITE 7: note = Methyl-L-phenylalanine
  SITE 10: note = Methyl-L-phenylalanine
XSXIRYXQTXIVGCG

SEQ ID NO: 13 - protein, 15 aa, unidentified
  SITE 1: note = D-phenylalanine
  SITE 7: note = Methyl-L-phenylalanine
  SITE 10: note = Methyl-L-phenylalanine
XSDIEYXQTXIVGCG

SEQ ID NO: 14 - protein, 15 aa, unidentified
  SITE 1: note = D-phenylalanine
  SITE 5: note = (S)-2-aminoheptanoic acid
  SITE 7: note = Methyl-L-phenylalanine
  SITE 10: note = Methyl-L-phenylalanine
XSDIXYXQTXIVGCG

SEQ ID NO: 15 - protein, 15 aa, unidentified
  SITE 1: note = D-phenylalanine
  SITE 7: note = Methyl-L-phenylalanine
  SITE 8: note = L-2-aminoadipic acid
  SITE 10: note = Methyl-L-phenylalanine
XSDIRYXXTXIVGCG

SEQ ID NO: 16 - protein, 15 aa, unidentified
  SITE 1: note = D-phenylalanine
  SITE 7: note = Methyl-L-phenylalanine
  SITE 8: note = 1-(carboxymethyl)-L-tryptophan
  SITE 10: note = Methyl-L-phenylalanine
XSDIRYXXTXIVGCG

SEQ ID NO: 17 - protein, 15 aa, unidentified
  SITE 1: note = D-phenylalanine
  SITE 7: note = Methyl-L-phenylalanine
  SITE 10: note = Methyl-L-phenylalanine
XSDIRYXVTXIVGCG

SEQ ID NO: 18 - protein, 15 aa, unidentified
  SITE 1: note = D-phenylalanine
  SITE 7: note = Methyl-L-phenylalanine
  SITE 8: note = (S)-2-aminoheptanoic acid
  SITE 10: note = Methyl-L-phenylalanine
XSDIRYXXTXIVGCG

SEQ ID NO: 19 - protein, 15 aa, unidentified
  SITE 1: note = D-phenylalanine
  SITE 7: note = Methyl-L-phenylalanine
  SITE 8: note = homo-L-tyrosine
  SITE 10: note = Methyl-L-phenylalanine
XSDIRYXXTXIVGCG

SEQ ID NO: 20 - protein, 15 aa, unidentified
  SITE 1: note = D-phenylalanine
  SITE 7: note = Methyl-L-phenylalanine
  SITE 10: note = Methyl-L-phenylalanine
XSDIRYXTTXIVGCG

SEQ ID NO: 21 - protein, 15 aa, unidentified
  SITE 1: note = D-phenylalanine
  SITE 7: note = Methyl-L-phenylalanine
  SITE 8: note = allo-threonine
  SITE 10: note = Methyl-L-phenylalanine
XSDIRYXXTXIVGCG

SEQ ID NO: 22 - protein, 15 aa, unidentified
  SITE 1: note = D-phenylalanine
  SITE 7: note = Methyl-L-phenylalanine
  SITE 8: note = L-citrulline
  SITE 10: note = Methyl-L-phenylalanine
XSDIRYXXTXIVGCG

SEQ ID NO: 23 - protein, 15 aa, unidentified
  SITE 1: note = D-phenylalanine
  SITE 7: note = Methyl-L-phenylalanine
  SITE 8: note = N6-(4-(carboxymethyl)piperazine-1-carbonyl)-L-lysine
  SITE 10: note = Methyl-L-phenylalanine
XSDIRYXXTXIVGCG

SEQ ID NO: 24 - protein, 15 aa, unidentified
  SITE 1: note = D-phenylalanine
  SITE 7: note = Methyl-L-phenylalanine
  SITE 10: note = (S)-2-(methylamino)hexanoic acid
XSDIRYXQTXIVGCG

SEQ ID NO: 25 - protein, 15 aa, unidentified
  SITE 1: note = D-phenylalanine
  SITE 7: note = Methyl-L-phenylalanine
  SITE 10: note = Methyl-L-phenylalanine
XSDIRYXQTXYVGCG

SEQ ID NO: 26 - protein, 15 aa, unidentified
  SITE 1: note = D-phenylalanine
  SITE 7: note = Methyl-L-phenylalanine
  SITE 10: note = Methyl-L-phenylalanine
  SITE 11: note = (S)-2-amino-3-(4-(carboxymethoxy)phenyl)propanoic acid
XSDIRYXQTXXVGCG

SEQ ID NO: 27 - protein, 15 aa, unidentified
  SITE 1: note = (R)-2-amino-3-(pyridin-4-yl)propanoic acid
  SITE 7: note = Methyl-L-phenylalanine
  SITE 10: note = Methyl-L-phenylalanine
  SITE 12: note = Methyl-L-valine
XSDIRYXVTXIXGCG

SEQ ID NO: 28 - protein, 15 aa, unidentified
  SITE 1: note = (R)-2-amino-3-(pyridin-3-yl)propanoic acid
  SITE 7: note = Methyl-L-phenylalanine
  SITE 10: note = Methyl-L-phenylalanine
  SITE 12: note = Methyl-L-valine
XSDIRYXVTXIXGCG

SEQ ID NO: 29 - protein, 15 aa, unidentified
  SITE 1: note = (R)-2-amino-3-(3-methoxyphenyl)propanoic acid
  SITE 7: note = Methyl-L-phenylalanine
  SITE 10: note = Methyl-L-phenylalanine
  SITE 12: note = Methyl-L-valine
XSDIRYXVTXIXGCG

SEQ ID NO: 30 - protein, 15 aa, unidentified
  SITE 1: note = (R)-2-amino-3-(4-methoxyphenyl)propanoic acid
  SITE 7: note = Methyl-L-phenylalanine
  SITE 10: note = Methyl-L-phenylalanine
  SITE 12: note = Methyl-L-valine
XSDIRYXVTXIXGCG

SEQ ID NO: 31 - protein, 15 aa, unidentified
  SITE 1: note = D-phenylalanine
  SITE 7: note = Methyl-L-phenylalanine
  SITE 10: note = Methyl-L-phenylalanine
  SITE 12: note = Methyl-L-valine
XNDIRYXVTXIXGCG

SEQ ID NO: 32 - protein, 15 aa, unidentified
  SITE 1: note = D-phenylalanine
  SITE 7: note = Methyl-L-phenylalanine
  SITE 10: note = Methyl-L-phenylalanine
  SITE 12: note = Methyl-L-valine
XDDIRYXVTXIXGCG

SEQ ID NO: 33 - protein, 15 aa, unidentified
  SITE 1: note = D-phenylalanine
  SITE 2: note = L-2-aminoadipic acid
  SITE 7: note = Methyl-L-phenylalanine
  SITE 10: note = Methyl-L-phenylalanine
  SITE 12: note = Methyl-L-valine
XXDIRYXVTXIXGCG

SEQ ID NO: 34 - protein, 15 aa, unidentified
  SITE 1: note = D-phenylalanine
  SITE 2: note = L-citrulline
  SITE 7: note = Methyl-L-phenylalanine
  SITE 10: note = Methyl-L-phenylalanine
  SITE 12: note = Methyl-L-valine
XXDIRYXVTXIXGCG

SEQ ID NO: 35 - protein, 15 aa, unidentified
  SITE 1: note = D-phenylalanine
  SITE 3: note = (2S)-2-amino-3-(oxan-4-yl)propanoic acid
  SITE 7: note = Methyl-L-phenylalanine
  SITE 10: note = Methyl-L-phenylalanine
  SITE 12: note = Methyl-L-valine
XSXIRYXVTXIXGCG

SEQ ID NO: 36 - protein, 15 aa, unidentified
  SITE 1: note = D-phenylalanine
  SITE 7: note = Methyl-L-phenylalanine
  SITE 10: note = Methyl-L-phenylalanine
  SITE 12: note = Methyl-L-valine
XSNIRYXVTXIXGCG

SEQ ID NO: 37 - protein, 15 aa, unidentified
  SITE 1: note = D-phenylalanine
  SITE 7: note = Methyl-L-phenylalanine
  SITE 10: note = Methyl-L-phenylalanine
  SITE 12: note = Methyl-L-valine
XSSIRYXVTXIXGCG

SEQ ID NO: 38 - protein, 15 aa, unidentified
  SITE 1: note = D-phenylalanine
  SITE 4: note = O-methyl-L-threonine
  SITE 7: note = Methyl-L-phenylalanine
  SITE 10: note = Methyl-L-phenylalanine
  SITE 12: note = Methyl-L-valine
XSDXRYXVTXIXGCG

SEQ ID NO: 39 - protein, 15 aa, unidentified
  SITE 1: note = D-phenylalanine
  SITE 7: note = Methyl-L-phenylalanine
  SITE 10: note = Methyl-L-phenylalanine
  SITE 12: note = Methyl-L-valine
XSDISYXVTXIXGCG

SEQ ID NO: 40 - protein, 15 aa, unidentified
  SITE 1: note = D-phenylalanine
  SITE 5: note = L-homoserine
  SITE 7: note = Methyl-L-phenylalanine
  SITE 10: note = Methyl-L-phenylalanine
  SITE 12: note = Methyl-L-valine
XSDIXYXVTXIXGCG

SEQ ID NO: 41 - protein, 15 aa, unidentified
  SITE 1: note = D-phenylalanine
  SITE 5: note = L-citrulline
  SITE 7: note = Methyl-L-phenylalanine
  SITE 10: note = Methyl-L-phenylalanine
  SITE 12: note = Methyl-L-valine
XSDIXYXVTXIXGCG

SEQ ID NO: 42 - protein, 15 aa, unidentified
  SITE 1: note = D-phenylalanine
  SITE 5: note = N6-carbamoyl-L-lysine
  SITE 7: note = Methyl-L-phenylalanine
  SITE 10: note = Methyl-L-phenylalanine
  SITE 12: note = Methyl-L-valine
XSDIXYXVTXIXGCG

SEQ ID NO: 43 - protein, 15 aa, unidentified
  SITE 1: note = D-phenylalanine
  SITE 5: note = (S)-2-amino-4-ureidobutanoic acid
  SITE 7: note = Methyl-L-phenylalanine
  SITE 10: note = Methyl-L-phenylalanine
  SITE 12: note = Methyl-L-valine
XSDIXYXVTXIXGCG

SEQ ID NO: 44 - protein, 15 aa, unidentified
  SITE 1: note = D-phenylalanine
  SITE 5: note = (S)-5-acetamido-2-aminopentanoic acid
  SITE 7: note = Methyl-L-phenylalanine
  SITE 10: note = Methyl-L-phenylalanine
  SITE 12: note = Methyl-L-valine
XSDIXYXVTXIXGCG

SEQ ID NO: 45 - protein, 15 aa, unidentified
  SITE 1: note = D-phenylalanine
  SITE 6: note = (S)-2-amino-3-(4-fluorophenyl)propanoic acid
  SITE 7: note = Methyl-L-phenylalanine
  SITE 10: note = Methyl-L-phenylalanine
  SITE 12: note = Methyl-L-valine
XSDIRXXVTXIXGCG

SEQ ID NO: 46 - protein, 15 aa, unidentified
  SITE 1: note = D-phenylalanine
  SITE 6: note = (S)-2-amino-3-(4-chlorophenyl)propanoic acid
  SITE 7: note = Methyl-L-phenylalanine
  SITE 10: note = Methyl-L-phenylalanine
  SITE 12: note = Methyl-L-valine
XSDIRXXVTXIXGCG

SEQ ID NO: 47 - protein, 15 aa, unidentified
  SITE 1: note = D-phenylalanine
  SITE 6: note = (S)-2-amino-3-(pyridin-4-yl)propanoic acid
  SITE 7: note = Methyl-L-phenylalanine
  SITE 10: note = Methyl-L-phenylalanine
  SITE 12: note = Methyl-L-valine
XSDIRXXVTXIXGCG

SEQ ID NO: 48 - protein, 15 aa, unidentified
  SITE 1: note = D-phenylalanine
  SITE 6: note = (S)-3-(2-amino-2-carboxyethyl)benzoic acid
  SITE 7: note = Methyl-L-phenylalanine
  SITE 10: note = Methyl-L-phenylalanine
  SITE 12: note = Methyl-L-valine
XSDIRXXVTXIXGCG

SEQ ID NO: 49 - protein, 15 aa, unidentified
  SITE 1: note = D-phenylalanine
  SITE 7: note = (S)-2-(methylamino)-3-(pyridin-3-yl)propanoic acid
  SITE 10: note = Methyl-L-phenylalanine
  SITE 12: note = Methyl-L-valine
XSDIRYXVTXIXGCG

SEQ ID NO: 50 - protein, 15 aa, unidentified
  SITE 1: note = D-phenylalanine
  SITE 7: note = (S)-2-(methylamino)-3-(pyridin-4-yl)propanoic acid
  SITE 10: note = Methyl-L-phenylalanine
  SITE 12: note = Methyl-L-valine
XSDIRYXVTXIXGCG

SEQ ID NO: 51 - protein, 15 aa, unidentified
  SITE 1: note = D-phenylalanine
  SITE 7: note = (S)-3-(2-carboxy-2-(methylamino)ethyl)benzoic acid
  SITE 10: note = Methyl-L-phenylalanine
  SITE 12: note = Methyl-L-valine
XSDIRYXVTXIXGCG

SEQ ID NO: 52 - protein, 15 aa, unidentified
  SITE 1: note = D-phenylalanine
  SITE 7: note = (S)-4-(2-carboxy-2-(methylamino)ethyl)benzoic acid
  SITE 10: note = Methyl-L-phenylalanine
  SITE 12: note = Methyl-L-valine
XSDIRYXVTXIXGCG

SEQ ID NO: 53 - protein, 15 aa, unidentified
  SITE 1: note = D-phenylalanine
  SITE 7: note = (S)-2-(methylamino)-3-(tetrahydro-2H-pyran-4-yl)propanoic acid
  SITE 10: note = Methyl-L-phenylalanine
  SITE 12: note = Methyl-L-valine
XSDIRYXVTXIXGCG

SEQ ID NO: 54 - protein, 15 aa, unidentified
  SITE 1: note = D-phenylalanine
  SITE 7: note = Methyl-L-phenylalanine
  SITE 8: note = (S)-2-amino-2-(tetrahydro-2H-pyran-4-yl)acetic acid
  SITE 10: note = Methyl-L-phenylalanine
  SITE 12: note = Methyl-L-valine
XSDIRYXXTXIXGCG

SEQ ID NO: 55 - protein, 15 aa, unidentified
  SITE 1: note = D-phenylalanine
  SITE 7: note = Methyl-L-phenylalanine
  SITE 8: note = (S)-2-amino-2-(1-(carboxymethyl)piperidin-4-yl)acetic acid
  SITE 10: note = Methyl-L-phenylalanine
  SITE 12: note = Methyl-L-valine
XSDIRYXXTXIXGCG

SEQ ID NO: 56 - protein, 15 aa, unidentified
  SITE 1: note = D-phenylalanine
  SITE 7: note = Methyl-L-phenylalanine
  SITE 8: note = (S)-2-amino-2-cyclobutylacetic acid
  SITE 10: note = Methyl-L-phenylalanine
  SITE 12: note = Methyl-L-valine
XSDIRYXXTXIXGCG

SEQ ID NO: 57 - protein, 15 aa, unidentified
  SITE 1: note = D-phenylalanine
  SITE 7: note = Methyl-L-phenylalanine
  SITE 8: note = (S)-2-amino-2-cyclohexylacetic acid
  SITE 10: note = Methyl-L-phenylalanine
  SITE 12: note = Methyl-L-valine
XSDIRYXXTXIXGCG

SEQ ID NO: 58 - protein, 15 aa, unidentified
  SITE 1: note = D-phenylalanine
  SITE 7: note = Methyl-L-phenylalanine
  SITE 8: note = O-methyl-L-threonine
  SITE 10: note = Methyl-L-phenylalanine
  SITE 12: note = Methyl-L-valine
XSDIRYXXTXIXGCG

SEQ ID NO: 59 - protein, 15 aa, unidentified
  SITE 1: note = D-phenylalanine
  SITE 7: note = Methyl-L-phenylalanine
  SITE 10: note = (S)-2-(methylamino)-3-(pyridin-3-yl)propanoic acid
  SITE 12: note = Methyl-L-valine
XSDIRYXVTXIXGCG

SEQ ID NO: 60 - protein, 15 aa, unidentified
  SITE 1: note = D-phenylalanine
  SITE 7: note = Methyl-L-phenylalanine
  SITE 10: note = (S)-2-(methylamino)-3-(pyridin-4-yl)propanoic acid
  SITE 12: note = Methyl-L-valine
XSDIRYXVTXIXGCG

SEQ ID NO: 61 - protein, 15 aa, unidentified
  SITE 1: note = D-phenylalanine
  SITE 7: note = Methyl-L-phenylalanine
  SITE 10: note = (S)-4-(2-carboxy-2-(methylamino)ethyl)benzoic acid
  SITE 12: note = Methyl-L-valine
XSDIRYXVTXIXGCG

SEQ ID NO: 62 - protein, 15 aa, unidentified
  SITE 1: note = D-phenylalanine
  SITE 7: note = Methyl-L-phenylalanine
  SITE 10: note = (S)-2-(methylamino)-3-(tetrahydro-2H-pyran-4-yl)propanoic acid
  SITE 12: note = Methyl-L-valine
XSDIRYXVTXIXGCG

SEQ ID NO: 63 - protein, 15 aa, unidentified
  SITE 1: note = D-phenylalanine
  SITE 7: note = Methyl-L-phenylalanine
  SITE 10: note = Methyl-L-phenylalanine
  SITE 11: note = O-methyl-L-threonine
  SITE 12: note = Methyl-L-valine
XSDIRYXVTXXXGCG

SEQ ID NO: 64 - protein, 15 aa, unidentified
  SITE 1: note = D-phenylalanine
  SITE 7: note = Methyl-L-phenylalanine
  SITE 10: note = Methyl-L-phenylalanine
  SITE 12: note = (S)-2-cyclohexyl-2-(methylamino)acetic acid
XSDIRYXVTXIXGCG

SEQ ID NO: 65 - protein, 15 aa, unidentified
  SITE 1: note = D-phenylalanine
  SITE 7: note = Methyl-L-phenylalanine
  SITE 10: note = Methyl-L-phenylalanine
  SITE 12: note = Methyl-L-valine
  SITE 13: note = D-alanine
XSDIRYXVTXIXXCG

SEQ ID NO: 66 - protein, 15 aa, unidentified
  SITE 1: note = D-phenylalanine
  SITE 7: note = Methyl-L-phenylalanine
  SITE 10: note = Methyl-L-phenylalanine
  SITE 12: note = Methyl-L-valine
  SITE 13: note = D-serine
XSDIRYXVTXIXXCG

SEQ ID NO: 67 - protein, 15 aa, unidentified
  SITE 1: note = D-phenylalanine
  SITE 3: note = (2S)-2-amino-3-(oxan-4-yl)propanoic acid
  SITE 7: note = Methyl-L-phenylalanine
  SITE 10: note = Methyl-L-phenylalanine
XSXIRYXVTXIVGCG

SEQ ID NO: 68 - protein, 15 aa, unidentified
  SITE 1: note = D-phenylalanine
  SITE 3: note = L-citrulline
  SITE 7: note = Methyl-L-phenylalanine
  SITE 10: note = Methyl-L-phenylalanine
  SITE 12: note = Methyl-L-valine
XSXIRYXVTXIXGCG

SEQ ID NO: 69 - protein, 15 aa, unidentified
  SITE 1: note = D-phenylalanine
  SITE 3: note = (2S)-2-amino-3-(oxan-4-yl)propanoic acid
  SITE 7: note = Methyl-L-phenylalanine
  SITE 10: note = Methyl-L-phenylalanine
  SITE 12: note = Methyl-L-valine
XSXIRYXVTXYXGCG

SEQ ID NO: 70 - protein, 15 aa, unidentified
  SITE 1: note = D-phenylalanine
  SITE 2: note = L-2-aminoadipic acid
  SITE 7: note = Methyl-L-phenylalanine
  SITE 10: note = (S)-2-(methylamino)-3-(pyridin-4-yl)propanoic acid
  SITE 12: note = Methyl-L-valine
XXDIRYXVTXIXGCG

SEQ ID NO: 71 - protein, 15 aa, unidentified
  SITE 1: note = D-phenylalanine
  SITE 2: note = L-2-aminoadipic acid
  SITE 7: note = (S)-3-(2-carboxy-2-(methylamino)ethyl)benzoic acid
  SITE 10: note = (S)-2-(methylamino)-3-(pyridin-4-yl)propanoic acid
  SITE 12: note = Methyl-L-valine
XXDIRYXVTXIXGCG

SEQ ID NO: 72 - protein, 15 aa, unidentified
  SITE 1: note = D-phenylalanine
  SITE 2: note = L-2-aminoadipic acid
  SITE 5: note = L-citrulline
  SITE 7: note = (S)-3-(2-carboxy-2-(methylamino)ethyl)benzoic acid
  SITE 10: note = (S)-2-(methylamino)-3-(pyridin-4-yl)propanoic acid
  SITE 12: note = Methyl-L-valine
XXDIXYXVTXIXGCG

SEQ ID NO: 73 - protein, 15 aa, unidentified
  SITE 1: note = D-phenylalanine
  SITE 2: note = L-2-aminoadipic acid
  SITE 5: note = L-citrulline
  SITE 7: note = (S)-3-(2-carboxy-2-(methylamino)ethyl)benzoic acid
  SITE 8: note = O-methyl-L-threonine
  SITE 10: note = (S)-2-(methylamino)-3-(pyridin-4-yl)propanoic acid
  SITE 12: note = Methyl-L-valine
  SITE 13: note = D-serine
XXDIXYXXTXIXXCG

SEQ ID NO: 74 - protein, 15 aa, unidentified
  SITE 1: note = D-phenylalanine
  SITE 7: note = Methyl-L-phenylalanine
  SITE 10: note = (S)-2-(methylamino)-3-(pyridin-4-yl)propanoic acid
  SITE 12: note = Methyl-L-valine
  SITE 13: note = D-serine
XSDIRYXVTXIXXCG

SEQ ID NO: 75 - protein, 15 aa, unidentified
  SITE 1: note = D-phenylalanine
  SITE 2: note = L-2-aminoadipic acid
  SITE 7: note = Methyl-L-phenylalanine
  SITE 10: note = (S)-2-(methylamino)-3-(pyridin-4-yl)propanoic acid
  SITE 12: note = Methyl-L-valine
  SITE 13: note = D-serine
XXDIRYXVTXIXXCG

SEQ ID NO: 76 - protein, 15 aa, unidentified
  SITE 1: note = D-phenylalanine
  SITE 3: note = L-citrulline
  SITE 7: note = Methyl-L-phenylalanine
  SITE 10: note = (S)-2-(methylamino)-3-(pyridin-4-yl)propanoic acid
  SITE 12: note = Methyl-L-valine
  SITE 13: note = D-serine
XSXIRYXVTXIXXCG

SEQ ID NO: 77 - protein, 15 aa, unidentified
  SITE 1: note = D-phenylalanine
  SITE 2: note = L-2-aminoadipic acid
  SITE 7: note = (S)-3-(2-carboxy-2-(methylamino)ethyl)benzoic acid
  SITE 10: note = (S)-2-(methylamino)-3-(pyridin-4-yl)propanoic acid
  SITE 12: note = Methyl-L-valine
  SITE 13: note = D-serine
XXDIRYXVTXIXXCG

SEQ ID NO: 78 - protein, 15 aa, unidentified
  SITE 1: note = D-phenylalanine
  SITE 2: note = L-2-aminoadipic acid
  SITE 5: note = L-citrulline
  SITE 7: note = (S)-3-(2-carboxy-2-(methylamino)ethyl)benzoic acid
  SITE 10: note = (S)-2-(methylamino)-3-(pyridin-4-yl)propanoic acid
  SITE 12: note = Methyl-L-valine
  SITE 13: note = D-serine
XXDIXYXVTXIXXCG

SEQ ID NO: 79 - protein, 15 aa, unidentified
  SITE 7: note = Methyl-L-phenylalanine
  SITE 12: note = (S)-1,2,3,4-tetrahydroisoquinoline-3-carboxylic acid
FRWDVRXSNWNXNCG

SEQ ID NO: 80 - protein, 15 aa, unidentified
  SITE 1: note = (S)-2-amino-3-(4-fluorophenyl)propanoic acid
  SITE 7: note = Methyl-L-phenylalanine
  SITE 12: note = (S)-1,2,3,4-tetrahydroisoquinoline-3-carboxylic acid
XRWDVRXSNWNXNCG

SEQ ID NO: 81 - protein, 15 aa, unidentified
  SITE 3: note = Methyl-L-tryptophan
  SITE 7: note = Methyl-L-phenylalanine
  SITE 12: note = (S)-1,2,3,4-tetrahydroisoquinoline-3-carboxylic acid
FRXDVRXSNWNXNCG

SEQ ID NO: 82 - protein, 15 aa, unidentified
  SITE 5: note = Methyl-L-valine
  SITE 7: note = Methyl-L-phenylalanine
  SITE 12: note = (S)-1,2,3,4-tetrahydroisoquinoline-3-carboxylic acid
FRWDXRXSNWNXNCG

SEQ ID NO: 83 - protein, 15 aa, unidentified
  SITE 6: note = Methyl-L-arginine
  SITE 7: note = Methyl-L-phenylalanine
  SITE 12: note = (S)-1,2,3,4-tetrahydroisoquinoline-3-carboxylic acid
FRWDVXXSNWNXNCG

SEQ ID NO: 84 - protein, 15 aa, unidentified
  SITE 7: note = Methyl-L-phenylalanine
  SITE 9: note = Methyl-L-asparagine
  SITE 12: note = (S)-1,2,3,4-tetrahydroisoquinoline-3-carboxylic acid
FRWDVRXSXWNXNCG

SEQ ID NO: 85 - protein, 15 aa, unidentified
  SITE 3: note = (S)-2-amino-3-(1H-pyrrolo[2,3-b]pyridin-3-yl)propanoic acid
  SITE 7: note = Methyl-L-phenylalanine
  SITE 12: note = (S)-1,2,3,4-tetrahydroisoquinoline-3-carboxylic acid
FRXDVRXSNWNXNCG

SEQ ID NO: 86 - protein, 15 aa, unidentified
  SITE 5: note = 1-(carboxymethyl)-L-tryptophan
  SITE 7: note = Methyl-L-phenylalanine
  SITE 12: note = (S)-1,2,3,4-tetrahydroisoquinoline-3-carboxylic acid
FRWDXRXSNWNXNCG

SEQ ID NO: 87 - protein, 15 aa, unidentified
  SITE 5: note = (S)-2-amino-3-cyclohexylpropanoic acid
  SITE 7: note = Methyl-L-phenylalanine
  SITE 12: note = (S)-1,2,3,4-tetrahydroisoquinoline-3-carboxylic acid
FRWDXRXSNWNXNCG

SEQ ID NO: 88 - protein, 15 aa, unidentified
  SITE 5: note = (S)-2-amino-3-(naphthalen-1-yl)propanoic acid
  SITE 7: note = Methyl-L-phenylalanine
  SITE 12: note = (S)-1,2,3,4-tetrahydroisoquinoline-3-carboxylic acid
FRWDXRXSNWNXNCG

SEQ ID NO: 89 - protein, 15 aa, unidentified
  SITE 5: note = (S)-2-amino-3-(5-phenylpyridin-3-yl)propanoic acid
  SITE 7: note = Methyl-L-phenylalanine
  SITE 12: note = (S)-1,2,3,4-tetrahydroisoquinoline-3-carboxylic acid
FRWDXRXSNWNXNCG

SEQ ID NO: 90 - protein, 15 aa, unidentified
  SITE 6: note = (S)-2-amino-6-morpholinohexanoic acid
  SITE 7: note = Methyl-L-phenylalanine
  SITE 12: note = (S)-1,2,3,4-tetrahydroisoquinoline-3-carboxylic acid
FRWDVXXSNWNXNCG

SEQ ID NO: 91 - protein, 15 aa, unidentified
  SITE 7: note = Methyl-L-phenylalanine
  SITE 8: note = 1-(carboxymethyl)-L-tryptophan
  SITE 12: note = (S)-1,2,3,4-tetrahydroisoquinoline-3-carboxylic acid
FRWDVRXXNWNXNCG

SEQ ID NO: 92 - protein, 15 aa, unidentified
  SITE 7: note = Methyl-L-phenylalanine
  SITE 8: note = homo-L-tyrosine
  SITE 12: note = (S)-1,2,3,4-tetrahydroisoquinoline-3-carboxylic acid
FRWDVRXXNWNXNCG

SEQ ID NO: 93 - protein, 15 aa, unidentified
  SITE 7: note = Methyl-L-phenylalanine
  SITE 8: note = allo-threonine
  SITE 12: note = (S)-1,2,3,4-tetrahydroisoquinoline-3-carboxylic acid
FRWDVRXXNWNXNCG

SEQ ID NO: 94 - protein, 15 aa, unidentified
  SITE 7: note = Methyl-L-phenylalanine
  SITE 9: note = L-2-aminoadipic acid
  SITE 12: note = (S)-1,2,3,4-tetrahydroisoquinoline-3-carboxylic acid
FRWDVRXSXWNXNCG

SEQ ID NO: 95 - protein, 15 aa, unidentified
  SITE 7: note = Methyl-L-phenylalanine
  SITE 9: note = (S)-2-amino-3-cyclohexylpropanoic acid
  SITE 12: note = (S)-1,2,3,4-tetrahydroisoquinoline-3-carboxylic acid
FRWDVRXSXWNXNCG

SEQ ID NO: 96 - protein, 15 aa, unidentified
  SITE 7: note = Methyl-L-phenylalanine
  SITE 9: note = homo-L-tyrosine
  SITE 12: note = (S)-1,2,3,4-tetrahydroisoquinoline-3-carboxylic acid
FRWDVRXSXWNXNCG

SEQ ID NO: 97 - protein, 15 aa, unidentified
  SITE 7: note = Methyl-L-phenylalanine
  SITE 9: note = (S)-2-amino-4-(1H-pyrrolo[2,3-b]pyridin-3-yl)butanoic acid
  SITE 12: note = (S)-1,2,3,4-tetrahydroisoquinoline-3-carboxylic acid
FRWDVRXSXWNXNCG

SEQ ID NO: 98 - protein, 15 aa, unidentified
  SITE 7: note = Methyl-L-phenylalanine
  SITE 9: note = N6-(4-(carboxymethyl)piperazine-1-carbonyl)-L-lysine
  SITE 12: note = (S)-1,2,3,4-tetrahydroisoquinoline-3-carboxylic acid
FRWDVRXSXWNXNCG

SEQ ID NO: 99 - protein, 15 aa, unidentified
  SITE 7: note = Methyl-L-phenylalanine
  SITE 10: note = (S)-2-amino-3-(1H-pyrrolo[2,3-b]pyridin-3-yl)propanoic acid
  SITE 12: note = (S)-1,2,3,4-tetrahydroisoquinoline-3-carboxylic acid
FRWDVRXSNXNXNCG

SEQ ID NO: 100 - protein, 15 aa, unidentified
  SITE 7: note = Methyl-L-phenylalanine
  SITE 12: note = (S)-1,2,3,4-tetrahydroisoquinoline-3-carboxylic acid
FRWDVRXSNWNXDCG

SEQ ID NO: 101 - protein, 15 aa, unidentified
  SITE 1: note = (S)-2-amino-3-(p-toluyl)propanoic acid
  SITE 7: note = Methyl-L-phenylalanine
  SITE 12: note = (S)-1,2,3,4-tetrahydroisoquinoline-3-carboxylic acid
XRWDVRXSNWNXNCG

SEQ ID NO: 102 - protein, 15 aa, unidentified
  SITE 1: note = (S)-2-amino-3-(m-toluyl)propanoic acid
  SITE 7: note = Methyl-L-phenylalanine
  SITE 12: note = (S)-1,2,3,4-tetrahydroisoquinoline-3-carboxylic acid
XRWDVRXSNWNXNCG

SEQ ID NO: 103 - protein, 15 aa, unidentified
  SITE 2: note = N6-carbamoyl-L-lysine
  SITE 7: note = Methyl-L-phenylalanine
  SITE 12: note = (S)-1,2,3,4-tetrahydroisoquinoline-3-carboxylic acid
FXWDVRXSNWNXNCG

SEQ ID NO: 104 - protein, 15 aa, unidentified
  SITE 3: note = (S)-2-amino-3-(1H-pyrrolo[3,2-c]pyridin-3-yl)propanoic acid
  SITE 7: note = Methyl-L-phenylalanine
  SITE 12: note = (S)-1,2,3,4-tetrahydroisoquinoline-3-carboxylic acid
FRXDVRXSNWNXNCG

SEQ ID NO: 105 - protein, 15 aa, unidentified
  SITE 3: note = (S)-2-amino-3-(1H-pyrrolo[2,3-b]pyridin-3-yl)propanoic acid
  SITE 7: note = Methyl-L-phenylalanine
  SITE 12: note = (S)-1,2,3,4-tetrahydroisoquinoline-3-carboxylic acid
FRXDVRXSNWNXNCG

SEQ ID NO: 106 - protein, 15 aa, unidentified
  SITE 3: note = (S)-2-amino-3-(1-methyl-1H-pyrrolo[2,3-b]pyridin-3-yl)propanoic acid
  SITE 7: note = Methyl-L-phenylalanine
  SITE 12: note = (S)-1,2,3,4-tetrahydroisoquinoline-3-carboxylic acid
FRXDVRXSNWNXNCG

SEQ ID NO: 107 - protein, 15 aa, unidentified
  SITE 3: note = (S)-2-amino-3-(5-methyl-1H-pyrrolo[2,3-b]pyridin-3-yl)propanoic acid
  SITE 7: note = Methyl-L-phenylalanine
  SITE 12: note = (S)-1,2,3,4-tetrahydroisoquinoline-3-carboxylic acid
FRXDVRXSNWNXNCG

SEQ ID NO: 108 - protein, 15 aa, unidentified
  SITE 3: note = (S)-2-amino-3-(naphthalen-1-yl)propanoic acid
  SITE 7: note = Methyl-L-phenylalanine
  SITE 12: note = (S)-1,2,3,4-tetrahydroisoquinoline-3-carboxylic acid
FRXDVRXSNWNXNCG

SEQ ID NO: 109 - protein, 15 aa, unidentified
  SITE 3: note = (S)-2-amino-3-(quinolin-4-yl)propanoic acid
  SITE 7: note = Methyl-L-phenylalanine
  SITE 12: note = (S)-1,2,3,4-tetrahydroisoquinoline-3-carboxylic acid
FRXDVRXSNWNXNCG

SEQ ID NO: 110 - protein, 15 aa, unidentified
  SITE 7: note = Methyl-L-phenylalanine
  SITE 12: note = (S)-1,2,3,4-tetrahydroisoquinoline-3-carboxylic acid
FRWEVRXSNWNXNCG

SEQ ID NO: 111 - protein, 15 aa, unidentified
  SITE 7: note = Methyl-L-phenylalanine
  SITE 12: note = (S)-1,2,3,4-tetrahydroisoquinoline-3-carboxylic acid
FRWNVRXSNWNXNCG

SEQ ID NO: 112 - protein, 15 aa, unidentified
  SITE 7: note = Methyl-L-phenylalanine
  SITE 12: note = (S)-1,2,3,4-tetrahydroisoquinoline-3-carboxylic acid
FRWQVRXSNWNXNCG

SEQ ID NO: 113 - protein, 15 aa, unidentified
  SITE 5: note = (S)-2-amino-2-cyclobutylacetic acid
  SITE 7: note = Methyl-L-phenylalanine
  SITE 12: note = (S)-1,2,3,4-tetrahydroisoquinoline-3-carboxylic acid
FRWDXRXSNWNXNCG

SEQ ID NO: 114 - protein, 15 aa, unidentified
  SITE 7: note = Methyl-L-phenylalanine
  SITE 12: note = (S)-1,2,3,4-tetrahydroisoquinoline-3-carboxylic acid
FRWDPRXSNWNXNCG

SEQ ID NO: 115 - protein, 15 aa, unidentified
  SITE 6: note = L-citrulline
  SITE 7: note = Methyl-L-phenylalanine
  SITE 12: note = (S)-1,2,3,4-tetrahydroisoquinoline-3-carboxylic acid
FRWDVXXSNWNXNCG

SEQ ID NO: 116 - protein, 15 aa, unidentified
  SITE 6: note = N6-carbamoyl-L-lysine
  SITE 7: note = Methyl-L-phenylalanine
  SITE 12: note = (S)-1,2,3,4-tetrahydroisoquinoline-3-carboxylic acid
FRWDVXXSNWNXNCG

SEQ ID NO: 117 - protein, 15 aa, unidentified
  SITE 6: note = (S)-2-amino-4-ureidobutanoic acid
  SITE 7: note = Methyl-L-phenylalanine
  SITE 12: note = (S)-1,2,3,4-tetrahydroisoquinoline-3-carboxylic acid
FRWDVXXSNWNXNCG

SEQ ID NO: 118 - protein, 15 aa, unidentified
  SITE 6: note = (S)-5-acetamido-2-aminopentanoic acid
  SITE 7: note = Methyl-L-phenylalanine
  SITE 12: note = (S)-1,2,3,4-tetrahydroisoquinoline-3-carboxylic acid
FRWDVXXSNWNXNCG

SEQ ID NO: 119 - protein, 15 aa, unidentified
  SITE 7: note = (S)-4-(2-carboxy-2-(methylamino)ethyl)benzoic acid
  SITE 12: note = (S)-1,2,3,4-tetrahydroisoquinoline-3-carboxylic acid
FRWDVRXSNWNXNCG

SEQ ID NO: 120 - protein, 15 aa, unidentified
  SITE 7: note = Methyl-L-tyrosine
  SITE 12: note = (S)-1,2,3,4-tetrahydroisoquinoline-3-carboxylic acid
FRWDVRXSNWNXNCG

SEQ ID NO: 121 - protein, 15 aa, unidentified
  SITE 7: note = (S)-2-(methylamino)-3-(p-toluyl)propanoic acid
  SITE 12: note = (S)-1,2,3,4-tetrahydroisoquinoline-3-carboxylic acid
FRWDVRXSNWNXNCG

SEQ ID NO: 122 - protein, 15 aa, unidentified
  SITE 7: note = (S)-3-(4-chlorophenyl)-2-(methylamino)propanoic acid
  SITE 12: note = (S)-1,2,3,4-tetrahydroisoquinoline-3-carboxylic acid
FRWDVRXSNWNXNCG

SEQ ID NO: 123 - protein, 15 aa, unidentified
  SITE 7: note = (S)-3-(2-carboxy-2-(methylamino)ethyl)benzoic acid
  SITE 12: note = (S)-1,2,3,4-tetrahydroisoquinoline-3-carboxylic acid
FRWDVRXSNWNXNCG

SEQ ID NO: 124 - protein, 15 aa, unidentified
  SITE 7: note = (S)-2-(methylamino)-3-(m-toluyl)propanoic acid
  SITE 12: note = (S)-1,2,3,4-tetrahydroisoquinoline-3-carboxylic acid
FRWDVRXSNWNXNCG

SEQ ID NO: 125 - protein, 15 aa, unidentified
  SITE 7: note = (S)-3-(3-chlorophenyl)-2-(methylamino)propanoic acid
  SITE 12: note = (S)-1,2,3,4-tetrahydroisoquinoline-3-carboxylic acid
FRWDVRXSNWNXNCG

SEQ ID NO: 126 - protein, 15 aa, unidentified
  SITE 7: note = Methyl-L-phenylalanine
  SITE 12: note = (S)-1,2,3,4-tetrahydroisoquinoline-3-carboxylic acid
FRWDVRXTNWNXNCG

SEQ ID NO: 127 - protein, 15 aa, unidentified
  SITE 7: note = Methyl-L-phenylalanine
  SITE 12: note = (S)-1,2,3,4-tetrahydroisoquinoline-3-carboxylic acid
FRWDVRXNNWNXNCG

SEQ ID NO: 128 - protein, 15 aa, unidentified
  SITE 7: note = Methyl-L-phenylalanine
  SITE 12: note = (S)-1,2,3,4-tetrahydroisoquinoline-3-carboxylic acid
FRWDVRXQNWNXNCG

SEQ ID NO: 129 - protein, 15 aa, unidentified
  SITE 7: note = Methyl-L-phenylalanine
  SITE 12: note = (S)-1,2,3,4-tetrahydroisoquinoline-3-carboxylic acid
FRWDVRXDNWNXNCG

SEQ ID NO: 130 - protein, 15 aa, unidentified
  SITE 7: note = Methyl-L-phenylalanine
  SITE 12: note = (S)-1,2,3,4-tetrahydroisoquinoline-3-carboxylic acid
FRWDVRXENWNXNCG

SEQ ID NO: 131 - protein, 15 aa, unidentified
  SITE 7: note = Methyl-L-phenylalanine
  SITE 12: note = (S)-1,2,3,4-tetrahydroisoquinoline-3-carboxylic acid
FRWDVRXSQWNXNCG

SEQ ID NO: 132 - protein, 15 aa, unidentified
  SITE 7: note = Methyl-L-phenylalanine
  SITE 12: note = (S)-1,2,3,4-tetrahydroisoquinoline-3-carboxylic acid
FRWDVRXSDWNXNCG

SEQ ID NO: 133 - protein, 15 aa, unidentified
  SITE 7: note = Methyl-L-phenylalanine
  SITE 12: note = (S)-1,2,3,4-tetrahydroisoquinoline-3-carboxylic acid
FRWDVRXSEWNXNCG

SEQ ID NO: 134 - protein, 15 aa, unidentified
  SITE 7: note = Methyl-L-phenylalanine
  SITE 10: note = (S)-2-amino-3-(1H-pyrrolo[2,3-c]pyridin-3-yl)propanoic acid
  SITE 12: note = (S)-1,2,3,4-tetrahydroisoquinoline-3-carboxylic acid
FRWDVRXSNXNXNCG

SEQ ID NO: 135 - protein, 15 aa, unidentified
  SITE 7: note = Methyl-L-phenylalanine
  SITE 10: note = (S)-2-amino-3-(1-methyl-1H-pyrrolo[2,3-b]pyridin-3-yl)propanoic acid
  SITE 12: note = (S)-1,2,3,4-tetrahydroisoquinoline-3-carboxylic acid
FRWDVRXSNXNXNCG

SEQ ID NO: 136 - protein, 15 aa, unidentified
  SITE 7: note = Methyl-L-phenylalanine
  SITE 10: note = (S)-2-amino-3-(5-methyl-1H-pyrrolo[2,3-b]pyridin-3-yl)propanoic acid
  SITE 12: note = (S)-1,2,3,4-tetrahydroisoquinoline-3-carboxylic acid
FRWDVRXSNXNXNCG

SEQ ID NO: 137 - protein, 15 aa, unidentified
  SITE 7: note = Methyl-L-phenylalanine
  SITE 12: note = (S)-1,2,3,4-tetrahydroisoquinoline-3-carboxylic acid
FRWDVRXSNWQXNCG

SEQ ID NO: 138 - protein, 15 aa, unidentified
  SITE 7: note = Methyl-L-phenylalanine
  SITE 11: note = (2S)-2-amino-4-(methylamino)-4-oxobutanoic acid
  SITE 12: note = (S)-1,2,3,4-tetrahydroisoquinoline-3-carboxylic acid
FRWDVRXSNWXXNCG

SEQ ID NO: 139 - protein, 15 aa, unidentified
  SITE 7: note = Methyl-L-phenylalanine
  SITE 12: note = (S)-6-chloro-1,2,3,4-tetrahydroisoquinoline-3-carboxylic acid
FRWDVRXSNWNXNCG

SEQ ID NO: 140 - protein, 15 aa, unidentified
  SITE 7: note = Methyl-L-phenylalanine
  SITE 12: note = (S)-7-hydroxy-1,2,3,4-tetrahydroisoquinoline-3-carboxylic acid
FRWDVRXSNWNXNCG

SEQ ID NO: 141 - protein, 15 aa, unidentified
  SITE 7: note = Methyl-L-phenylalanine
  SITE 12: note = (S)-7-chloro-1,2,3,4-tetrahydroisoquinoline-3-carboxylic acid
FRWDVRXSNWNXNCG

SEQ ID NO: 142 - protein, 15 aa, unidentified
  SITE 7: note = Methyl-L-phenylalanine
  SITE 12: note = (S)-1,2,3,4-tetrahydroisoquinoline-3-carboxylic acid
FRWDVRXSNWNXQCG

SEQ ID NO: 143 - protein, 15 aa, unidentified
  SITE 7: note = Methyl-L-phenylalanine
  SITE 12: note = (S)-1,2,3,4-tetrahydroisoquinoline-3-carboxylic acid
  SITE 13: note = (2S)-2-amino-4-(methylamino)-4-oxobutanoic acid
FRWDVRXSNWNXXCG

SEQ ID NO: 144 - protein, 15 aa, unidentified
  SITE 7: note = Methyl-L-phenylalanine
  SITE 12: note = (S)-1,2,3,4-tetrahydroisoquinoline-3-carboxylic acid
  SITE 13: note = (2S)-2-amino-4-(dimethylamino)-4-oxobutanoic acid
FRWDVRXSNWNXXCG

SEQ ID NO: 145 - protein, 15 aa, unidentified
  SITE 3: note = (S)-2-amino-3-(1H-pyrrolo[2,3-b]pyridin-3-yl)propanoic acid
  SITE 7: note = Methyl-L-phenylalanine
  SITE 10: note = (S)-2-amino-3-(1H-pyrrolo[2,3-b]pyridin-3-yl)propanoic acid
  SITE 12: note = (S)-1,2,3,4-tetrahydroisoquinoline-3-carboxylic acid
FRXDVRXSNXNXNCG

SEQ ID NO: 146 - protein, 15 aa, unidentified
  SITE 3: note = (S)-2-amino-3-(5-methyl-1H-pyrrolo[2,3-b]pyridin-3-yl)propanoic acid
  SITE 7: note = Methyl-L-phenylalanine
  SITE 10: note = (S)-2-amino-3-(1H-pyrrolo[2,3-b]pyridin-3-yl)propanoic acid
  SITE 12: note = (S)-1,2,3,4-tetrahydroisoquinoline-3-carboxylic acid
FRXDVRXSNXNXNCG

SEQ ID NO: 147 - protein, 15 aa, unidentified
  SITE 3: note = (S)-2-amino-3-(quinolin-4-yl)propanoic acid
  SITE 7: note = Methyl-L-phenylalanine
  SITE 10: note = (S)-2-amino-3-(1H-pyrrolo[2,3-b]pyridin-3-yl)propanoic acid
  SITE 12: note = (S)-1,2,3,4-tetrahydroisoquinoline-3-carboxylic acid
FRXDVRXSNXNXNCG

SEQ ID NO: 148 - protein, 15 aa, unidentified
  SITE 3: note = (S)-2-amino-3-(1H-pyrrolo[2,3-b]pyridin-3-yl)propanoic acid
  SITE 5: note = (S)-2-amino-2-cyclobutylacetic acid
  SITE 7: note = Methyl-L-phenylalanine
  SITE 10: note = (S)-2-amino-3-(1H-pyrrolo[2,3-b]pyridin-3-yl)propanoic acid
  SITE 12: note = (S)-1,2,3,4-tetrahydroisoquinoline-3-carboxylic acid
FRXDXRXSNXNXNCG

SEQ ID NO: 149 - protein, 15 aa, unidentified
  SITE 3: note = (S)-2-amino-3-(1H-pyrrolo[2,3-b]pyridin-3-yl)propanoic acid
  SITE 7: note = Methyl-L-phenylalanine
  SITE 10: note = (S)-2-amino-3-(1H-pyrrolo[2,3-b]pyridin-3-yl)propanoic acid
  SITE 12: note = (S)-1,2,3,4-tetrahydroisoquinoline-3-carboxylic acid
FRXDPRXSNXNXNCG

SEQ ID NO: 150 - protein, 15 aa, unidentified
  SITE 3: note = (S)-2-amino-3-(1H-pyrrolo[2,3-b]pyridin-3-yl)propanoic acid
  SITE 6: note = (S)-2-amino-6-morpholinohexanoic acid
  SITE 7: note = Methyl-L-phenylalanine
  SITE 10: note = (S)-2-amino-3-(1H-pyrrolo[2,3-b]pyridin-3-yl)propanoic acid
  SITE 12: note = (S)-1,2,3,4-tetrahydroisoquinoline-3-carboxylic acid
FRXDVXXSNXNXNCG

SEQ ID NO: 151 - protein, 15 aa, unidentified
  SITE 3: note = (S)-2-amino-3-(1H-pyrrolo[2,3-b]pyridin-3-yl)propanoic acid
  SITE 7: note = (S)-4-(2-carboxy-2-(methylamino)ethyl)benzoic acid
  SITE 10: note = (S)-2-amino-3-(1H-pyrrolo[2,3-b]pyridin-3-yl)propanoic acid
  SITE 12: note = (S)-1,2,3,4-tetrahydroisoquinoline-3-carboxylic acid
FRXDVRXSNXNXNCG

SEQ ID NO: 152 - protein, 15 aa, unidentified
  SITE 3: note = (S)-2-amino-3-(1H-pyrrolo[2,3-b]pyridin-3-yl)propanoic acid
  SITE 7: note = (S)-3-(2-carboxy-2-(methylamino)ethyl)benzoic acid
  SITE 10: note = (S)-2-amino-3-(1H-pyrrolo[2,3-b]pyridin-3-yl)propanoic acid
  SITE 12: note = (S)-1,2,3,4-tetrahydroisoquinoline-3-carboxylic acid
FRXDVRXSNXNXNCG

SEQ ID NO: 153 - protein, 15 aa, unidentified
  SITE 3: note = (S)-2-amino-3-(1H-pyrrolo[2,3-b]pyridin-3-yl)propanoic acid
  SITE 7: note = Methyl-L-phenylalanine
  SITE 10: note = (S)-2-amino-3-(1H-pyrrolo[2,3-b]pyridin-3-yl)propanoic acid
  SITE 12: note = (S)-1,2,3,4-tetrahydroisoquinoline-3-carboxylic acid
FRXDVRXENXNXNCG

SEQ ID NO: 154 - protein, 15 aa, unidentified
  SITE 3: note = (S)-2-amino-3-(1H-pyrrolo[2,3-b]pyridin-3-yl)propanoic acid
  SITE 7: note = Methyl-L-phenylalanine
  SITE 10: note = (S)-2-amino-3-(1H-pyrrolo[2,3-b]pyridin-3-yl)propanoic acid
  SITE 12: note = (S)-1,2,3,4-tetrahydroisoquinoline-3-carboxylic acid
FRXDVRXSEXNXNCG

SEQ ID NO: 155 - protein, 15 aa, unidentified
  SITE 3: note = (S)-2-amino-3-(1H-pyrrolo[2,3-b]pyridin-3-yl)propanoic acid
  SITE 7: note = Methyl-L-phenylalanine
  SITE 10: note = (S)-2-amino-3-(5-methyl-1H-pyrrolo[2,3-b]pyridin-3-yl)propanoic acid
  SITE 12: note = (S)-1,2,3,4-tetrahydroisoquinoline-3-carboxylic acid
FRXDVRXSNXNXNCG

SEQ ID NO: 156 - protein, 15 aa, unidentified
  SITE 3: note = (S)-2-amino-3-(1H-pyrrolo[2,3-b]pyridin-3-yl)propanoic acid
  SITE 7: note = Methyl-L-phenylalanine
  SITE 10: note = (S)-2-amino-3-(1H-pyrrolo[2,3-b]pyridin-3-yl)propanoic acid
  SITE 12: note = (S)-7-chloro-1,2,3,4-tetrahydroisoquinoline-3-carboxylic acid
FRXDVRXSNXNXNCG

SEQ ID NO: 157 - protein, 15 aa, unidentified
  SITE 3: note = (S)-2-amino-3-(1H-pyrrolo[2,3-b]pyridin-3-yl)propanoic acid
  SITE 7: note = Methyl-L-phenylalanine
  SITE 10: note = (S)-2-amino-3-(1H-pyrrolo[2,3-b]pyridin-3-yl)propanoic acid
  SITE 12: note = (S)-1,2,3,4-tetrahydroisoquinoline-3-carboxylic acid
  SITE 13: note = (2S)-2-amino-4-(methylamino)-4-oxobutanoic acid
FRXDVRXSNXNXXCG

SEQ ID NO: 158 - protein, 15 aa, unidentified
  SITE 3: note = (S)-2-amino-3-(1H-pyrrolo[2,3-b]pyridin-3-yl)propanoic acid
  SITE 7: note = Methyl-L-phenylalanine
  SITE 10: note = (S)-2-amino-3-(1H-pyrrolo[2,3-b]pyridin-3-yl)propanoic acid
  SITE 12: note = (S)-1,2,3,4-tetrahydroisoquinoline-3-carboxylic acid
FRXDVRXSNXNXDCG

SEQ ID NO: 159 - protein, 15 aa, unidentified
  SITE 3: note = (S)-2-amino-3-(1H-pyrrolo[2,3-b]pyridin-3-yl)propanoic acid
  SITE 7: note = Methyl-L-phenylalanine
  SITE 10: note = (S)-2-amino-3-(1H-pyrrolo[2,3-b]pyridin-3-yl)propanoic acid
  SITE 12: note = (S)-1,2,3,4-tetrahydroisoquinoline-3-carboxylic acid
FRXDVRXEEXNXNCG

SEQ ID NO: 160 - protein, 15 aa, unidentified
  SITE 3: note = (S)-2-amino-3-(1H-pyrrolo[2,3-b]pyridin-3-yl)propanoic acid
  SITE 7: note = Methyl-L-phenylalanine
  SITE 10: note = (S)-2-amino-3-(1H-pyrrolo[2,3-b]pyridin-3-yl)propanoic acid
  SITE 12: note = (S)-1,2,3,4-tetrahydroisoquinoline-3-carboxylic acid
FRXDVRXEEXNXDCG

SEQ ID NO: 161 - protein, 15 aa, unidentified
  SITE 3: note = (S)-2-amino-3-(1H-pyrrolo[2,3-b]pyridin-3-yl)propanoic acid
  SITE 7: note = (S)-3-(2-carboxy-2-(methylamino)ethyl)benzoic acid
  SITE 10: note = (S)-2-amino-3-(1H-pyrrolo[2,3-b]pyridin-3-yl)propanoic acid
  SITE 12: note = (S)-1,2,3,4-tetrahydroisoquinoline-3-carboxylic acid
FRXDVRXEEXNXDCG

SEQ ID NO: 162 - protein, 15 aa, unidentified
  SITE 3: note = (S)-2-amino-3-(1H-pyrrolo[2,3-b]pyridin-3-yl)propanoic acid
  SITE 6: note = (S)-2-amino-6-morpholinohexanoic acid
  SITE 7: note = (S)-3-(2-carboxy-2-(methylamino)ethyl)benzoic acid
  SITE 10: note = (S)-2-amino-3-(1H-pyrrolo[2,3-b]pyridin-3-yl)propanoic acid
  SITE 12: note = (S)-1,2,3,4-tetrahydroisoquinoline-3-carboxylic acid
FRXDVXXEEXNXDCG

SEQ ID NO: 163 - protein, 15 aa, unidentified
  SITE 3: note = (S)-2-amino-3-(1H-pyrrolo[2,3-b]pyridin-3-yl)propanoic acid
  SITE 7: note = (S)-3-(2-carboxy-2-(methylamino)ethyl)benzoic acid
  SITE 10: note = (S)-2-amino-3-(1H-pyrrolo[2,3-b]pyridin-3-yl)propanoic acid
  SITE 12: note = (S)-1,2,3,4-tetrahydroisoquinoline-3-carboxylic acid
FRXDVRXSEXNXDCG

SEQ ID NO: 164 - protein, 14 aa, unidentified
  SITE 1: note = D-phenylalanine
  SITE 7: note = Methyl-L-phenylalanine
  SITE 10: note = Methyl-L-phenylalanine
XSDIRYXQTXIVGC

SEQ ID NO: 165 - protein, 14 aa, unidentified
  SITE 7: note = Methyl-L-phenylalanine
  SITE 12: note = (S)-1,2,3,4-tetrahydroisoquinoline-3-carboxylic acid
FRWDVRXSNWNXNC